European Patent Application EP 4 728 882 A1, published April 22, 2026. Title: Lactobacillus Paracasei L-30 Straim and uses thereof. Applicant: NEOREGEN BIOTECH. Application KR 10-024-0143193, filed October 18, 2024. The sequence listing filed with the application follows.

SEQUENCE LISTING (1 sequence)

SEQ ID NO: 1 - DNA, 1511 bp, Lactobacillus paracasei
  source 1..1511: mol_type = genomic DNA
tggctcaggatgaacgctggcggcgtgcctaatacatgcaagtcgaacgagttctcgttgatgatcggtgcttgcaccgagattcaacatggaacgagtggcggacgggtgagtaacacgtgggtaacctgcccttaagtgggggataacatttggaaacagatgctaataccgcatagatccaagaaccgcatggttcttggctgaaagatggcgtaagctatcgcttttggatggacccgcggcgtattagctagttggtgaggtaatggctcaccaaggcgatgatacgtagccgaactgagaggttgatcggccacattgggactgagacacggcccaaactcctacgggaggcagcagtagggaatcttccacaatggacgcaagtctgatggagcaacgccgcgtgagtgaagaaggctttcgggtcgtaaaactctgttgttggagaagaatggtcggcagagtaactgttgtcggcgtgacggtatccaaccagaaagccacggctaactacgtgccagcagccgcggtaatacgtaggtggcaagcgttatccggatttattgggcgtaaagcgagcgcaggcggttttttaagtctgatgtgaaagccctcggcttaaccgaggaagcgcatcggaaactgggaaacttgagtgcagaagaggacagtggaactccatgtgtagcggtgaaatgcgtagatatatggaagaacaccagtggcgaaggcggctgtctggtctgtaactgacgctgaggctcgaaagcatgggtagcgaacaggattagataccctggtagtccatgccgtaaacgatgaatgctaggtgttggagggtttccgcccttcagtgccgcagctaacgcattaagcattccgcctggggagtacgaccgcaaggttgaaactcaaaggaattgacgggggcccgcacaagcggtggagcatgtggtttaattcgaagcaacgcgaagaaccttaccaggtcttgacatcttttgatcacctgagagatcaggtttccccttcgggggcaaaatgacaggtggtgcatggttgtcgtcagctcgtgtcgtgagatgttgggttaagtcccgcaacgagcgcaacccttatgactagttgccagcatttagttgggcactctagtaagactgccggtgacaaaccggaggaaggtggggatgacgtcaaatcatcatgccccttatgacctgggctacacacgtgctacaatggatggtacaacgagttgcgagaccgcgaggtcaagctaatctcttaaagccattctcagttcggactgtaggctgcaactcgcctacacgaagtcggaatcgctagtaatcgcggatcagcacgccgcggtgaatacgttcccgggccttgtacacaccgcccgtcacaccatgagagtttgtaacacccgaagccggtggcgtaacccttttagggagcgagccgtctaaggtgggacaaatgattaggggtgaagtcgtaac